European Patent Specification EP 4 008 344 B1, published December 6, 2023. Title: CORE/SHELL STRUCTURE PLATFORM FOR IMMUNOTHERAPY. Applicant: The Methodist Hospital SHEN, Haifa. The sequence listing filed with the application follows.

SEQUENCE LISTING (10 sequences)

SEQ ID NO: 1 - protein, 9 aa, Homo sapiens
TEVVRRCPH

SEQ ID NO: 2 - protein, 9 aa, Homo sapiens
TEVVHRCPH

SEQ ID NO: 3 - protein, 8 aa, Homo sapiens
TLEDSSGN

SEQ ID NO: 4 - protein, 8 aa, Homo sapiens
TDEDSSGN

SEQ ID NO: 5 - protein, 9 aa, Homo sapiens
GNREEKNRE

SEQ ID NO: 6 - protein, 9 aa, Homo sapiens
GNRENKNRE

SEQ ID NO: 7 - protein, 10 aa, Homo sapiens
QEKLKDETQK

SEQ ID NO: 8 - protein, 10 aa, Homo sapiens
QEKLKDKTQK

SEQ ID NO: 9 - protein, 9 aa, Homo sapiens
NHYKIYNLC

SEQ ID NO: 10 - protein, 9 aa, Homo sapiens
NHYNIYNLC